European Patent Application EP 4 137 582 A1, published February 22, 2023. Title: Rolling Circle Reverse Transcription of Circular RNA. Applicant: NEW ENGLAND BIOLABS, INC. The sequence listing filed with the application follows.

SEQUENCE LISTING (87 sequences)

SEQ ID NO: 1 - protein, 299 aa, synthetic construct
  REGION 1..299: note = Synthetic construct
MMNDGNDWIVDIDLEKFFDTVNHDKLMTIIGRTIKDGDVISIIRKYLVSGIMIDDEYEDSIVGTPQGGNLSPLLANIMLNELDKEMEKRGLNFVRYADDCIIMVGSEMSANRVMRNISRFIEEKLGLKVNMTKSKVDRPSGLKYLGFGFYFDTRAHQFKAKPHAKSVAKFKKRMKELTCRSWGVSNSYKVEKLNQLIRGWINYFKIGNMKRLCKELDSRIRYRLRMCIWKHWKTPQNRAKKLMKLDVPRWAAFKIAYCGDKYASLAHNGWVHKAISLKRLTSFGLVSMLDYYTERCVKC

SEQ ID NO: 2 - protein, 370 aa, synthetic construct
  REGION 1..370: note = Synthetic construct
MIRNGKYKPNPVRRVEIPKETKGEFRKIGVPTVVDRVIQQAITQELTPIYEEQFSENSFGFRPKRGAHGALKQCQKNVNDGYVYVVDMDLEKFFDTVSQSKLIEVLSRTIKDGRLISLIHKYLNAGVIANGMFERTEIGIPQGGPLSPLLSNVMLNELDKELERRGHRFVRYADDCMIFCKSKKSAERTLENILPFIEGKLFLKVNTMKTKVAHISKVKYLGYSFYRYKGKCRFRVHPKSVSKMKDKIRELTDRNNGMSNVIREERYQQYVRGWVEYFRLADMKSLLKTTDEWARRRIRAVYWKQWKKIKTRYRMLKALGMEHWKALELAWSRKGYWRMAQVLNQVFSNKIIAKLGYTSLLDYYLIVYEN

SEQ ID NO: 3 - protein, 427 aa, synthetic construct
  REGION 1..427: note = Synthetic construct
MRTGAIDELQELRRKIYLTAKSEKRKCFWGLFCHVTKIETLDKAYKLARENNGSAGVDGVTFADIERYGTYNFIKEIREELINGTYLPTRNRKVEIPKSNGKTRTLGIGTIKDRVVQGALKLILEPIFEADFSECSYGFRPKKNQHQAVNRVAKGIVRGFTKVIDVDLTAYFDNINHKILMDKIALRVNDSKIMRLIKLMLKINGKVGVPQGSVISPLFSNIYLNAIDRMFEKAKQGTSRKGYENMEYCRYADDTVILVNGHEAVDWLVSKSYRRLREELAKLKINLNVEKTKIVDMSQGETFGFLGFDFRLVKSKGKKMVLLKPKKKKVTELISKVKTHLVQSRNKTVTEMIEELNPILRGWVNYYRIGHCSRTLTYIKIWVERKVRRFARKAQKKFGFGWKEWSSEIIYGKWGLFSDYQVRYFSS

SEQ ID NO: 4 - protein, 428 aa, synthetic construct
  REGION 1..428: note = Synthetic construct
MIKTSIELQELRRRIYIKAKAEKDWKFWGLYIHVTKMETLAEAYKLAKGNNGAPGIDGVTFEDIENEGAGQFLKKIQEELTSETYLPMKNRIKDIPKGNGKTRTLGIPTIRDRVVQGALKLILEPIFEADFQDGSYGYRPKRTAHQAVERTAKAVIQGKTQVIDVDLSSYFDNVQHHILLGKVAKRINDRKVMRLLKLILKANGKIGLPQGGLISPLLSNLYLNEIDKMLEKAKEFTKKKDGYIHIEYVRYADDLVILIDGYHKWNRLMEFTMFRLKQEFEKIGVKINTEKTKIVNLLHGEIFSFLGFDYRRTKTKSGKWGVRKTPKMKARTKLLEKIKGIFKSQKSQPLDKVIKLINPILRGWVNYFRIGNSSQCFGYVKDWIQKKIRRHLMRARKLKGFGWDRWSNKWLYEKLNLYGDYKIRYFQG

SEQ ID NO: 5 - protein, 446 aa, synthetic construct
  REGION 1..446: note = Synthetic construct
MNVKTNDILGTVRYEPLEKAQELCEKLYLAAKNSETRRFHAIYDKVYRMDILNSAWNQVKANKGTKGIDNESISDILMKGEDIVISEIHQNLKERKYRPKQVERVYIPKPDGRMRPLGIPTIRDRIVQTATKHLIEPIFEADFIDCSYGFRPNRCAHEALEEIRKTMNAGYTIVLDADIKGFFDNIDHDKLLEFVHRRISDRRILKLIRKWLKCGIMDSGIVKESDMGTPQGGVISPLLANIYLHEFDKFWTQQTRVKGKLVRYADDFVIMFRTEKEAELGLKLIKAKMEELGLELNEDKTKIVDTRGGKEGFDFLGFHHRMTKSWKYKRYYAQKRPGDKSVKSIKTKIRNFLGQRAILNRSIDEVVKEINPVIRGWMNYFRFGNSADKFTQIDRYLHERLALWWSKKHQKSGRRWKSDFTWEKFKECGIQLLSGNVLYWSYYSNA

SEQ ID NO: 6 - protein, 389 aa, synthetic construct
  REGION 1..389: note = Synthetic construct
MKEITERRYYTLKDKITKIRNMKVAAKHVLDKGGSAGVDRIDTVEFKENYSIHMRELYREFLEDRYQPKPALRVFIPKSDGRQRPLGIPTVKDRIAQAAVRGILEPIYEKEFCDCSFGFRKGKSQMDAINQIEEYKEQGYKWVLDADIKGFFDNIDHKLLIEFIKQKVTDGWVIEIIKLWLTMGVMKDGKYIPTEKGTPQGGVISPLLANIFLHEFDKVMTERGYKLVRYADDFVVMTKSKRKAKRAYEVVKEIITEKLKLELHPEKTVITNFGEGFVFLGFEFIAWRYKRPRKKSLEKFKDKVRKVTKRNQPWKVDSIIKRLNAKIYGWANYFGHGNVKTLFRSLDEWIRMRLRSYIEKKKAVMNQNKRIPNSFFRKKGLVSLLTRLS

SEQ ID NO: 7 - protein, 427 aa, synthetic construct
  REGION 1..427: note = Synthetic construct
MKTDNTLLEEMLSDTNLELAFTQVKRNKGASGVDGMEVAELKDYLDKHLEEIKDSIRNKTYKPQPVRRVEIPKPDGGIRNLGVPTVLDRFVQQAIAQVLIPIYEPIFSDNSFGFRPNRCCEMAIIKALEYMNEGYQWIVDIDLEKFFDTVNHDKLISLVMKDVKSGEIVSLIRKYLVSGIMIDNEYKESVVGTPQGGNLSPLLSNIVLNELDKEMEARGLRFTRYADDCIILVGSSKAADRVMENISKFIEKKLGLKVNMTKSKVSKPNDIKYLGFGFYYDSFSSMWKAKPHEKSIATLQTKLRRLTNRSWSVSWEYRILKIRQLVNGWINYYRIGNFIKVCRKLDAQIRFRIRMYLWKKWKTIGNREKQLRKLGALPWQAKTWANSRKSYARCASTFLRTRITNDLLYRKGLPSMVAQYQLKHISV

SEQ ID NO: 8 - protein, 508 aa, synthetic construct
  REGION 1..508: note = Synthetic construct
MIISEMQHKLATWAASDPTRQFTRLLRLIVNRDWLAEAARIVLASNGARTPGIDGIDKHKMQRGLDDKLDQLQNDLLQGTYCPQPVKRIYIKKANGKLRPLGIPTLTDRIVQRAMLMVMDPIWESDFHRCSYGFRPERSVHHAVRTVKIQLQDGSDTKGRWVIEGDLASYFDTVHHKLLLKCVRRRIADNRFVDLLWRILKAGHVDKGLFRASSEGVPQGGVLSPLLSNIMLHEFDMWMEGNYLNKKVRKDRWAWNFGIQQGRPITIRENREWKPAVAFSRYADDFVVIVKGNKAHAEAIREQCRMFLEGKLKLTLNMEKTHITHVNDGFVFLGHRIIRKRGKTGRMSVVTTIPYEKAKAFAHKLSKALSGDHDLSKVDMVDRLNRKLSGWAAFYKFTDNTARTFQRIDRVVFWKLAHWLAQKYRSRIKPLMRNWCRAPEKGKAKTWVLFGISEQGNRVGKALHRLVGSPKMQFRWRNPETNPYIKREENRSTITSRYRDVAMAMGRA

SEQ ID NO: 9 - protein, 509 aa, synthetic construct
  REGION 1..509: note = Synthetic construct
MRPLGISSSDDKLVEEVIKMILESIYDPTFSNYSHGFRPGRSCHTALLQLQQNFTGVKWFVEGDIKSYFDTIDHHSLVNILRRRIKDEAFIELIWKFLNAGYMENWEYNATFSGIAQGSGISPILANIYLNEFDRFMEDYKKGFDKGMGRKRNNEYSRKQSYRQRCKAKIRKEWDGYSDTEKQEAVRQLAELKRAFQKIPMGDPMDTGYKRIQYVRYADDFLIGVIGSKEDAEKIKSDIGRFFEETLKLELSAEKTLITNSDDKARFLGYDVTVCNDRALKKAKGKGTVKAYTGKIKLYLPKEKWVGKLLGYGVLKIVSRAGEKEVWKPLQRNDYIFLPVHEMVRKYNAQIRGIYNYYRLASNVSVLNKFHYVMEYSLYKTVAAKYRITMTKAKLKYTKNKEFKVPYKTQKGIKYAVLYNEGFRRVKYALGSYADIIPEYEQMNKPKELFFRYKANVCEMCGAYVPAVKVYQVKSMNDLDVNTEWGAIMNRKKRKTLVVCGDCYDRIHK

SEQ ID NO: 10 - protein, 470 aa, synthetic construct
  REGION 1..470: note = Synthetic construct
MNVTNDRFKDRQLHIEDYRQMVSAEQKEYAEVFAYQRITENNDIIIDFWTENLMELILRKDNFNKAYKKVKSNKGAGGIDGMQVDNLLPYLRENQDELVQQIKLGKYKPNPVRRVEIPKEEKGKVRMLGIPTVVDRVIQQAMAQELTPIYEEQFSDSSFGFRPNRGQHDALKRCQKYVEEGYVYVVSMDLEKFFDTVNHSKLIEVLSRTIKDGRVIALIHKYLYAGVVRSGLFERTGEGFPQGGPLSPLLGNIMLNELDKELEQRGHKFVRYADDVVIFCKSKKSAERTLDNIVPYVEGKLFLKVNRAKTTISHVSKIKYLGYAFYRYKGKCRFRVHPKSVMKMKDKLRVLTNKSTGWDNDYRRQKLTEFVRGWINYFSMADMRGLMGEVDEWLRRRIRAIYWKQWKKVKTRYRILKALKLPEWKVHELANCRKGYWRATIMLNSVLTNKIIARLGYISMSDYYLKICEN

SEQ ID NO: 11 - protein, 441 aa, synthetic construct
  REGION 1..441: note = Synthetic construct
METNTEEGLTPKLTQLRAKLNFKAKQEPNFRFYTLYGHICNMEVLETAWKQVLKNRGTCGYDGVTLEDVKLRGVNEFLEEIRKSLVFRTYRADPVKRVYIPKSDGSLRPLGIPTVKDRVVQMALLLIIEPIFEADFLDCSYGFRPDKSTHQAIDAMVQAINEGKHEIYDADLEKYFNSIPHDKLIKAVEKRIVDNRVLNLIKMWLKAPIWEKGKPMDRNNVGVQQGGVISPILSNLYLHWFDKIFCSSKGPREWANAVLIRYADDIVIMAKFIGPKIKEWIQKVIEERFCLKINPAKTKIVKLKDNKAFVNFIGFTIRILRSGKVQIQPKKEAIKKAKLRIRELTSVKWGYLEIVKVIKRLNLFLVGWGKYFNKGSPSDAYQEINWYVEQRLRNFLERRSQKGYKKPKIIKWHACLKGMGLYTLTRSSLDKCRKPFKRRFM

SEQ ID NO: 12 - protein, 324 aa, synthetic construct
  REGION 1..324: note = Synthetic construct
MAVLLVTGPIFEVDLFRWQYGFRTGVDAKMALRRIHFGIVDRGARDVVDADLSDYFDTIPHGDLMRCVARRIADGSVLSVIRDWLNAPVIERTSNGERQSTEAKDSHRGTPQGGVISPLLANLYFRRFMLAWYGHGYADKYQAEIVNYADDFVILCREGRGEGAMEAMRHLMGKLGLTVNEKKTRLVKLPDERFDFLGYTVGRFYGLGGRPYWGTRPSKKSIKRLKDAVHDATTRRWNALDVESRVTELNPLLRGWAGYFNQGPVTRIYEDLDRYVARRLRVWLMRKRGKTGTGYRQYSDQFLYESLGLIRLRTLAANRSNAKV

SEQ ID NO: 13 - protein, 432 aa, synthetic construct
  REGION 1..432: note = Synthetic construct
MTKASISLQELRRKIYRKAKIEKQWRFWGLYCHVCKKEVLREAYRLAKANDGAPGNDGKSFEDIEAEGVEGFLEGIGQELLNRTYRPLPNRKVEIPKGNGKTRILGIPTVKDRVVQGALKLLLEPIFEADFKECSYGYRPKRHAHQAIDRVTKGILYGLTRVVDVDLSGYFDNIRHHILLEKIARRVQDDDIMHLVKLILKANGKKGVPQGGIISPLLSNLYLNEVDEMMERAREVTRSKGYENLDFIRYADDMVILVHWHPKEDWILQKVQKRHKEELDKLEVEMNLEKTKVVDLKKGGSFSFLGFDFRLTRNREGKAYVSKTPRKKKCIEIGKRVRAVLKANWNKPLKEVIQAVDAIIRGWVNYFRIGNSNSAFNKVRDYLEMKVRKFVLRRKKLKGFGWKMWSREEIYGKWGLYNDYRIRYVYPKANSS

SEQ ID NO: 14 - protein, 462 aa, synthetic construct
  REGION 1..462: note = Synthetic construct
MQTKLHRWAVADHGRRFDDVYNFVSDPATLVVALQRVAGNAGARTAGVDGVTAVHVSMAGPEVFLDHVRFLLKAGTFRPLPVREKMIPKTGGKLRRLGIPTITDRVVQAALKLVLEPIFEADFRPCSYGFRPNRRAHDAIAEIHHLATAGYRWVLDADIEACFDRIDHPALMGRVRARVKDKRVLTLVKAFLKAGIMTELGERNETTSGTPQGGILSPLLANIALSVLDEFFAEQWAAAGTGQQRRQRRAKGLATWQLVRYADDFLVLVHGNQEHVEDLRDQVSTVLATMGLRLSESKTRIAHLADGVDFLGFRIVWQRKRGTSKWHVYTFIADKPVQALKRKIKSLTRRLSHMSYRETLVRINYIQRGWANYFKHAVAKHTFSHLQNFIWWRVINWVMRRNRMTWRAIQRWLRTPQGWRPIVFDGVELFKIAKVSVTRYRYRGTKIPNPWQPTPTSPPPTA

SEQ ID NO: 15 - protein, 390 aa, synthetic construct
  REGION 1..390: note = Synthetic construct
MCANRGAPGVDGVTVDAVETSGVDAFLQDLSQRLRTHTYRPSVLRRVQIPKPGRPGEFRPLSIPTVADRVVMTAAKLVLEPVFEAQFTEASYGFRPKRSAIDACEAVRVAANQRREWVLEADIRDCFGTIDHEALMAQVARRVVDRPMLKLIRAWLRMGVLEGGVTSPTGAGTPQGSPISPLLANIALHVLDEAWQNEGCRLGVLVRYADDFVVLSPTEQRAEQARELAARVLERLGMRLHPEKTGIVRLTRGGQGFDFLGFHHRKMESWKWRGRYYLQRWPSARAMRVLRDKVRAATARSKTERPVSAVVADLNPVLRGWAAYFRNGNSGRKFNVVDGYVHERLAIFASAKHRLAGRNWTARFTYGWITRLGVYRLTGNVHRATAHASR

SEQ ID NO: 16 - protein, 484 aa, synthetic construct
  REGION 1..484: note = Synthetic construct
MEGAKSNTVSAIDGRQRKLGGQQGQTADGHLGMVGAELQEYPEAPTHMRIDPERKLDTKPDLLERICDRNNMRQAYVKVARNGGAGGVDGMSVKELDTWLHDNYDQLVLRILAGKYRPQPVRRVKIPKEEKGKLRLLGIPTVIDRMVQQAAVQVLTPIYEPMFSDASFGFRPNRSAHDALLRIKELADARDVWICSIDLERFFDTVNQSKLIQVMSNVVKDGRVVSLMHRFLKAGVMVDGVVMPTDEGTPQGGPLSPLLANVLLNELDRELERRGHHFVRYADDLIILKRSRKAAERAMGTVTKFIEGRLFLKVNRDKSYVAHIASHDPEVKYLGYGFFRYSGELHFRVHSKSAAKLKAKVKEVTSRSNGWSLDYRRKRLSWLVNGWVSYFRLADMTKLLRSVDEWLRRRIRCVYWKCWKKISTKYKALMKLGVSRNLAWQWANSRKAYWRIAGSAILARALNNTKLDELGWEFLYQRCLLVKC

SEQ ID NO: 17 - protein, 771 aa, synthetic construct
  REGION 1..771: note = Synthetic construct
MIAENLLEQFLSTSNFLTAYRRIASKKAAGGLDGITVEEFGHRLDQHITKLQKDIRERRYIPQPAAVTYIPKFNEENEWRELGLPSVADKVVQAAMLEVVEPLAEKMFLDCSYAYRPGTGHYKAIRRVENSLNNRKKTWVVQRDIDNFFDTVDHNRLMEQFSALVQGEPTMVELVALWCRMGLVEKNGRWRNVQAGIRQGGVISPLLANLYLHPLDVFATKLGVDWIRYADDYVILGESQEEVVSSDVQIVEFLKDSLGLMLNRDESSPKHIDEGFTFLGVRFCGKERAIDTKKIKKMKKKIRWLLAQKMVKTPEEVISKLTNQVESWQRYYSFLNPTRQFSEIDCFIEKEFLTLATSKIQTGKWDRIPPQGLSFPSLIADGKRDGFKKWEGLWAQAIKTVETDDVNHDTARINHSVEKKISRKRQKCRKESGESGNLIVTTPGHFVGKRGERIVVMSKQRIVSELPVVRLSGLTLSGRGVSISGDVVELCMKKDVYIHFVDNLGKIIAVVGPPGGSSGEVSLLQITERDKEKGLTLAKMFILGKVKNQFALLKYYFKYPLNRENGFGKIFVERRQFLSDGIEKIKNATVLSDPETFRQQMMGWEGAFGAAYWEIVGHLFRNGVQFSGRVRHGATDLVNSALNYGYGILYGDCLNAVIRTGLNPMAGFLHSYQTGKPTLIYDLIEEFRPFAVDRGIFTMLNRGERLEQGDDGMLATETRKKISKSVISRLSNEVWFHGRRLTLREVIQEQAYNIKRHLSDKAQYHPFLGRW

SEQ ID NO: 18 - protein, 379 aa, synthetic construct
  REGION 1..379: note = Synthetic construct
MAVHSIDRNTWLTKLERIKLLSSKNQDIKFNNLGHIIDLKMLEEQYKELDSKKAIGMDGITKEDYGKKLKANLLSLLTRIRKGQYQAKPARIVKIPKEDGGKRPLVISCFEDKIIESAVSKILNSVFEPIFLKYSYGFRPKLNAHDALRELNRLTYNFNKGAIVEIDITKCFNTIKHCELMEFLRKRISDKKFLRLIMKLIETPIIENGTIVTNKEGCRQGSIVSPILANVFLHYVIDSWFAKISEENLIGQTGMVRYADDMVFVFESEADAKRFYDVLPKRLNKYGLNINEAKSQMIKSGRDHAANLAKQGKKIASYNFLGFTCYWGKSRFGTTWRLKYTSRRDRFTEKLKGLRKYLRGQLNTLDKTQTLSQVIRVIR

SEQ ID NO: 19 - protein, 470 aa, synthetic construct
  REGION 1..470: note = Synthetic construct
MNVTESRFKNRQLHIEDYLQMVSAEQKEYAEVFDYSKITEKSGVITDYWTNNLLDLILRKDNLNNAYKQVKKNKGKGGNDGMQVDELLPFLRENQDTLIRKIREGKYKPNPVRRVEIPKETEGEFRKLGVPTVVDRVIQQAIAQELSPVYEKQFSENSFGFRPKRGAHDALRQCQKNVNDGYVYVVDMDLEKFFDTVCQSKLIEVLSRTIKDGRVISLIHKYLNAGVIAKGMFERTEVGMPQGGPLSPLLSNVMLNELDKELESRGHRFVRYADDCMIFCKSRKSAERTLKNIIPFIEGKLFLKVNRKKTEVSHISKVKYLGYSFYRYKGKCRFRVHSKSVVKMKNRIRELTDRNKGISNEVREKRYQEYVRGWVEYFRLADMKEFLRKTDEWARRRIRAVYWKQWKKIKTKYRMLKALGLEDWKAKELANSRKGYWRMAKVLNQIFSKKIIAKLGYTSMLDYYLIICEN

SEQ ID NO: 20 - protein, 470 aa, synthetic construct
  REGION 1..470: note = Synthetic construct
MNVTESRFKNRQLHIEDYLQMVSAEQREYAEVFDYSKITEKSGVITDYWTNNLLELILRKDNLNNAYKQVKRNRGKGGIDGMQVDELLPFLRENQETLIQEIKGGKYKPNPVRRVEIPKETKGEYRKLGVPTVVDRVIQQAIAQELSPIFEEQFSENSFGFRPKRGAHDALRQCQKNVNDGYVYVVDMDLEKFFDTVCQSKLIEVLSRTIKDGRVISLIHKYLNAGVIANGKFERTEVGMPQGGPLSPLLSNIMLNELDKELERREDRFVRYADDCMIFCKSRKSAERTLKNIIPFIEGKLFLKVNRKKTEVAHISKVKYLGYTFYRYKGKCRFRVHQKSVVKMRNKIRELTDRNKGISNAERERKYQEYVRGWVEYFRLADMKGLLKITDEWARRRIRAVYWKQWKKIKTKYRMLKALGMEHWKAKELACSRKGYWRMAKVLNQIFSKKIIAKLGYTSMLDYYLVVCEN

SEQ ID NO: 21 - protein, 470 aa, synthetic construct
  REGION 1..470: note = Synthetic construct
MDSKDMQRLQTTQQRGYPLNREMEFQKTTEVHSISSASEDGRNEVQRYTSKMLEMIVERGNMEAAYKRVVANKGSHGVDGMEVDELLPYLKENWATIKQQLLEGKYKPQPVRRVEISKPDGGVRLLGIPTALDRLIQQAIAQILNRVYNHTFSDSSYGFRPGRSAKDAIKAAEAYINEGYTWVVDMDLEKFFDRVNHDIIMSKLEKRIGDKRVLKLIRRYLESGVMINGIKVSTEEGTPQGGPLSPLLANIMLDELDKELEKRGHKFCRYADDCNIYVKSRSAGNRVMKSIKKFIESKLKLKINEAKSAVDRPWRRKFLGFSFYTKENEVRIRIHEKSIKRFKEKVREITNRNKGISMENRIKRLNQITTGWVNYFGLADAKSIMKTLDEWIRRRLRACIWKQWKKIKTKHDNLVKLGVEEQKAWEYANTRKGYWRISNSPILNKTLTNKYFESIGYKSLSQRYLIVHNS

SEQ ID NO: 22 - protein, 610 aa, synthetic construct
  REGION 1..610: note = Synthetic construct
MRIPKVVMDNLVEMSKRDENYVFERIYRNLYNEEFFLEAYAKLAKKEGNMTEGTDGKTIDGMSIDRIRKLIEQLKDESYQPNPSRREYIPKKPTGQRPLGIPSMDDKLVQEVARRILEGLYEPIFRDSSHGFRPNLSCQTAVDKIQKTFTGVKWFVEGDIKGFFDNIDHHTLINLLRKRIKDERFIRLIWKFLKAGYLEDWVYHKTFSGTPQGGVISPLLANTYLHELDKYMEQYAEEFNKGKKRKRTHDYRALEWQLTKMKKSDEEWDLMSTSEKKEHTKAYKALIKKRNEMNATDPFDTDFRRINYVRYADDFLVGVIGSKEDAEKTKQDIKAFLSNKLKLELSVEKTLITHAHKEKARFLGFDIVTSYSTQPTRNKDGKLQRQNNGKVKLYVPKEKWVNKLLDRNILRINGNDWKMVHRPELINNDDLEIISIYDAELRGFYEYYKIANNVSVLNKMAYIMEYSMYKTFARKYKISVRKVIDKFSVNGVFTVQYETKKGMRSKTLISSFTRVEKASTESKIDNLPNGWVYSGITSLIDRMKARVCEYCGATDVDLEMHHVRKLKDLKKKRSLQKWEVIMIARNRRQLALCARGQGNDCHMKLHKGQL

SEQ ID NO: 23 - protein, 448 aa, synthetic construct
  REGION 1..448: note = Synthetic construct
MYFAKETLAGHVGLDKLMQTSLRGIRQKAKENEKHRFQNLYQLLNEDTLMEAWKELNKKASAGVDEITAKEFKLNLRANIKEIVSNLKEKRYRTKLVRRVNIPKGKNESRPLGIPALSDKLVQRAVAKILEVIYEEDFLDCSYGYRPKIGAHKGIKDLTKELQFNKYSYIVEADIKGFFNNINHEWLIRMIEERVDDSALVGLIRKWLKAGILDANHLVIHPATGTPQGGIISPILANIYLHYALDLWFEKGVKRRCEGEAYLCRYADDFVCAFRYKKDADRFYKALGKRLRKFELELAEEKTNIISFSRFRKVENTHFDFLGFEFRWGVSLKGKDIIKRCTSKKKLRASLQNFKEWCKENRNNRLRKITEMLNKKLRGYFNYYGLIGNYESLWKFYTIAIETLYKWLNRRSQRKSFNWSEFTRLMKWYGVLKPKIVESSDHQLEFQY

SEQ ID NO: 24 - protein, 463 aa, synthetic construct
  REGION 1..463: note = Synthetic construct
MKNSKEMRKLQKTSYKEDWTWQVEVELQETMGVHSISTAFESGKDDGKLYTNNLLEKILDSENLRLAFRRVKSNKGSHGVDGMKVDELPQYLKQNIISLKKSILEGTYRPHPVRRVEIPKPDGGIRLLGIPTVVDRMIQQAVAQVLTPIFEKTFSENSYGFRPKRDAKQAIRKAKEYMEQGYKWVVDIDLAKYFDTVNHDKLMALVAREIKDKRVLKLIRLFLQSGVLINGVVIETEEGCPQGGPLSPLLSNIMLTELDRELEKRGHKFCRYADDNNIYVKSKKSGDRVMHSITEFIENKLKLKVNKDKSAVDRPWKRKFLGFSFYQWYGKIGIRVHEKSINKFKAKIRNITSRSNAWDMNYRMLKLRQCIVGWLNYFRIADIARLTKELDEWTRRRLRMCFWKQWKKIKTKHDNLKNLGIKESKAWEFANTRKSYWRIANSPILASTLTNSYLEKNRIYKYS

SEQ ID NO: 25 - protein, 427 aa, synthetic construct
  REGION 1..427: note = Synthetic construct
MDTSSLMEQVLSKDNLNAAYLQVVRNKGAAGVDGMTVEELGAYLSENGESIREKLRTRKYKPQPVRRVEIPKPEGGTRKLGVPTVVDRFVQQAVAQVLTPIFEEQFHDHSYGFRPNRCAQQAVLKALEMMNDGHSWVVDIDLAKFFDTVDHDKLMTIFGRTIKDGDVISVVRKFLVSGVMIDDEYEDTIVGTPQGGNISPLLANVMLNEVDKELEARGLDFVRYADDLIIMVGSRQAADRVMKSITRFIEERLGLKVNGEKSKVDKPKGIKYLGFGFYYDSFAKGYKARPHPKAAAKFREQMKKLTCRSWGVSNGYKVKKLNQLIRGWINYFKIGSMKGLCERLDSQIRYRLRMCIWKHWKTPQNRAKNLIKLGISRKYAWSTAYTGARIAYVCQRGAMNVAVTKERLTRFGLVSMSDYYAERRVTC

SEQ ID NO: 26 - protein, 427 aa, synthetic construct
  REGION 1..427: note = Synthetic construct
MDTSSLMEQILSKDNLNAAFLQVVRNKGAAGVDGMEYTELKDYLSENGETIKEQLRTRKYKPKPVRRVEIPKSDGGVRNLGVPTVTDRFVQQAIAQVLTPIFEEQFHEHSYGFRPNRCAQQAVIKALEMMNDGHSWIVDIDLAKFFDTVDHDKLMTIFGRTIKDGDVISIVRKFLVSGIMIGDEYEDSIIGTPQGGNISPLLANIMLNELDKELEARGLDFVRYADDCIIMVGSRQAAERVMKSVTRFIEDRLGLKVNATKSKIDKPKGIKYLGFGFYYDSFAKEYRAKPHAKSIVKFKARMKELTCRSWGVDNAYKVKKLNELIRGWINYFKIGSMKGLCAKLDSNIRFRLRMCIWKQWKTPQNRAKNLIKLGISRKFAWSTAYYGAHIAHVCQGGAMNMAVTKERLTRFGLVSMLDYYVERRVTC

SEQ ID NO: 27 - protein, 427 aa, synthetic construct
  REGION 1..427: note = Synthetic construct
MDTSSLMEQILSSGNLNRAYLQVVRNKGAEGVDGMKYTELKEHLEKNGEIIKEQLRTRKYKYQPVRRVEIPKPDGGVRNLGVPTVTDRFIQQAIAQVLTPIYEEQFHEHSYGFRPNRCAQQAILTALDMMNDGNDWIVDIDLEKFFDTVNHDKLMTIIGRTIKDGDVISIIRKYLVSGIMIDDEYEDSIVGTPQGGNLSPLLANIMLNELDKEMEKRGLNFVRYADDCIIMVGSEMSANRVMRNISRFIEEKLGLKVNMTKSKVDRPSGLKYLGFGFYFDTRAHQFKAKPHAKSVAKFKKRMKELTCRNWGVSNSYKVEKLNQLIRGWINYFKIGSMKTLCRKLDGNIRYRLRMCIWKHWKTPQNRAKNLMKFDVPRWAAFKIAYCGDRYARLAHNGWIQKAISTKGLTSFGLVSMLDYYTERCVTC

SEQ ID NO: 28 - protein, 427 aa, synthetic construct
  REGION 1..427: note = Synthetic construct
MDTSSLMEQILSSENLNRAYLQVVRNKGAEGVDGMKYTELKEHLEKNGDIIREQLRTRKYKPQPVRRVEIPKPDGGVRNLGVPTVTDRFIQQAIAQVLTPIYEEQFHDHSYGFRPNRCAQQAILTALDMMNDGNDWIVDIDLEKFFDTVNHDKLMTIIGRTIKDGDVISIVRKYLVSGIMIYDEYEDSIVGTPQGGNLSPLLANIMLNELDKEMEKRGLNFVRYADDCIIMVGSEVSANRVMRNISRFIEEKLGLKVNMTKSKVDKPQGLKYLGFGFYFDSRAHQFKAKPHAKSVAKFKKRMKELTSRSWGVSNSYKVEKLNQLIRGWINYFKIGSMKTLCKEMDSRIRFRLRMCIWKHWKTTQNRIKNLMKLGVDKDTAWITAYTGKRIAYVCQRRVMNFAINKERLTRFGLVSMLDYYTERCVTC

SEQ ID NO: 29 - protein, 427 aa, synthetic construct
  REGION 1..427: note = Synthetic construct
MDTSSLMEQILSKDNLNTAYLQVVRNKGAEGVDGMTYTELKEHLEKNGEIIREQLRTRKYKPQPVRRVEIPKPDGGVRNLGVPTVTDRFIQQATAQVLTPIYEEQFHDHSYGFRPNRCAQQAVIKALEMMNDGYDWIVDIDLEKFFDTVNHDKLMTLIGRTIKDGDVISIIRKFLVSGIMVDDEYKDSVIGTPQGGNLSPLLANVMLNELDKEMEQRGLNFVRYADDSIIMVGSEMSARRVMRNLAKFIEEKLGLKVNMTKSKVDRPRGLKYLGFGFYFDSRARQFKAKPHARSVVKFKAKMRQLTCRSWGISNSYKVKKLNELIRGWINYFKIGSMKTLCKEMDSQIRYRLRMCIWKHWKTPQNRAKNLMKLDVPRWAAFKIAYCGDRYARLAHNGWVQKAISNKRLTSFGLVSMLDYYTDRCVTC

SEQ ID NO: 30 - protein, 432 aa, synthetic construct
  REGION 1..432: note = Synthetic construct
MRGKGETSVELLETILSNQNMNEAYLRVYKNKDASGVDGVTVDELKQYLKENKDELRQRIRTRKYQPQAALRVEIPKENGKMRKLGIPTVVDRVVQQAIHQILSPIFEKQFSEFSYGFRPKRSCEMAIVKSLEFLNAGYEWIVDIDLERFFDTVHHDKLMRIISNTISDGDVISLIRKYLVSGVMVNGKYEETSVGTPQGGNLSPLLSNIMLNELDKELESRELQFVRYADDALIFVKSEKAASRVMKSIVRFIEKNLGLIVNTEKSKISRPEDLKFLGFGYYYNSKDERYQTKPHPISVQKLQRKLRHLTNRNWSVPLDYRILKLKQVIFGWVNYFRITNMKGVMKQVDKKLRSRIRVIIWKQWKIPKKQIKSLVQLGIPEEEAKGLTYCRKGYRYIGLSKVVQRAMSNQRLKKRGVPSSLERYLKVRTAI

SEQ ID NO: 31 - protein, 470 aa, synthetic construct
  REGION 1..470: note = Synthetic construct
MEMEQRGEQSISFSRVLIAEKTTSAVPNRERVVNSSETERNERMDTSSLMEQILSKENLNTAYLQVVRNKGAEGVDEMKYTELKEHLAKNGEIIKEQLRTRKYKPQPVRRVEIPKSDGGVRNLGVPTVTDRLVQQAIAQVLTPIYEEQFHDHSYGFRPNRCAQQAIITALDMMNDGYDWIVDIDLEKFFDTVNHDKLMTLIGKTIKDGDVISIIRKFLVSGIMVDDEYKESVIGTPQGGNLSPLLANIMLNELDKEMEQRGLNFVRYADDCIIMVGSEMSAKRVMRNLTKFIEEKLGLKVNMTKSKVDRPNGLKYLGFGFYFDSRAHQFKAKPHEKSVAKFKTKMKQLTCRSWGVSNTYKVQKLNELIRGWINYFKIGSMKTLCAKMDSNIRYRLRMCIWKHWKTSQNREKNLVKLGIDRNTARRVAYTGARIAYVCNKGAVNVAINNKRLASFGLISMLDYYTERCVTC

SEQ ID NO: 32 - protein, 438 aa, synthetic construct
  REGION 1..438: note = Synthetic construct
MVKSSETERKERMDTSNLMEQILSSDNLNRAYLQVVRNKGAEGVDGMKYTELKEHLAKNGEIIKEQLRTRKYKPQPVRRVEIPKPDGGVRNLGVPTVTDRFVQQAIAQVLTPIYEEQFHDHSYGFRPNRCAQQAILTALDMMNDGNDWIVDIDLEKFFDTVNHDKLMTLIGRTIKDGDVISIVRKYLVSGIMIDDEYENSVIGTPQGGNLSPLLANIMLNELDKEMEKRGLNFARYADDCIIMVGSEMSANRVMRNISRFIEEKLGLKVNMTKSKVDKPQGLKYLGFGFYFDSRAHQYKAKPHAKSVEKFKKRMKELTCRSWGVSNSYKVEKLNQLIRGWVNYFKIGSMKHLCREMDKHIRFRLRMCIWKQWKTPQNRAKNLMKLGVPQWAAKRTSYAKGFARVCRGSDVCQAISNKRLTSFGLVSMLDYYTERCVTC

SEQ ID NO: 33 - protein, 425 aa, synthetic construct
  REGION 1..425: note = Synthetic construct
MEEQGIFIERILSNENMNRAYKQVKKNKGAAGIDGMECADLLSHLKVNGQQLRESIRNQSYKPMPVKRVEIPKADGSKRKLGIPTVTDRMVQQAAAQVLTPIYERKFHENSYGFRPGKSAQKAVLKAVEYMNEGYNWVVDIDLEKFFDTVEHDKLISVLNKEIKDGKILSLIRKFLVSGVMVGEQIEETEIGTPQGGNISPLLANILLNELDWELESRGLKFARYADDCIIFVKSEKAAARVMESVTKYVENVLRLKVNRGKSKIGRPTEIQYLGFAFYYQFQEKKYKIKVPKKSLDKVMKKVRKLTSRKWGVSNSYKAQKIAEVVRGWINYFKIGSILTATRRLDTVIRYRFRMCIWKHWKNPKTRYKNLVKLGVSKKNAKSAAGFHGYARVCRTETICYAMSNARLKKFGLLSAEEYFCQTRC

SEQ ID NO: 34 - protein, 424 aa, synthetic construct
  REGION 1..424: note = Synthetic construct
MELLEQILRNQNMNEAYLRVYKNKGASGIDGVTVDELKQYLKENKDELRQRIRTRKYQPQAALRVEIPKENGKMRKLGIPTVVDRVVQQAIHQVLSPIFEKQFSEFSYGFRPKRSCEMAIIKSLEFLNDGHDWVVDIDLERFFDTVHHDKLMRIIANTIDDGDVISLIRKYLVSGVMVKGKYEETPVGTPQGGNLSPLLSNIMLNELDKELEGRGLRFVRYADDSLIFVKSEKAADRVMKSIVRFIEDKLGLIVNSEKSKISRPKELKFLGFGYYYDGKNKRYQVKPHLSSIQKFQRKLRKLTKRNWSVSLDYRILKLKQVIIGWVNYFRIGNMKNATERIDMKLRSRIRVIIWKQWKVPRKQIKSLTQLGIPKEEAKGLTYCRKGYRYIGLSKVIQRAISNKRLKQRGLPSALEHYLKVHTVI

SEQ ID NO: 35 - protein, 426 aa, synthetic construct
  REGION 1..426: note = Synthetic construct
MDTSSLMEQILSRDNLNAAYLQVVRNKGAEGVDGMKYTELKGHLEKNGEIIREQLRTRKYTPQPVRRVEIPKPDGGVRNLGVPTVTDRFVQQAIAQVLTPVYEEQFHDHSYGFRPNRCAQQAIITALDRMNDGYDWIVDIDLEKFFDTVNHDKLMTLMGKTIKDGEVISIIRKFPASGIKEDDEYRESVIGTRQGGNLSPLLANIMRNELDKEMEQRGMNFVRYADDCINMVGSEMSAKRVMRNITRFIEEKLGLKVNTTKSKVDKPQGIKYLGYGFYFDSRAHQYKAKPHAKSAAKFKARMKQLTCRSWGVSNIYKVQKLNELIRGWINYYKIGSMKTICARLDGSIRYRIRMCIWKHWKTPQNRARNLKKLGVPEWAARRTAYAKGYARVCRASDVCEAINNKRLASFGLISMLDYYTERCVTC

SEQ ID NO: 36 - protein, 424 aa, synthetic construct
  REGION 1..424: note = Synthetic construct
MELLEQILSNKNMNEAYIRVYKNKGASGVDGVTVDELKQYLKENKDELRQRIRTRKYQPQAALRVEIPKENGKMRKLGIPTVVDRVVQQAIHQVLSPIFEEQFSEFSYGFRPKRSCEMAIIKSLEFLNDEHDWVVDIDLERFFDTVHHDKLMRIISNTIKDGNVISLIRKYLVSGVMVNGKYEDTPVGTPQGGNLSPLLSNIMLNELDKELEKRGLRFVRYADDALIFVKSEKAANRVMSTIVRFIEEKLGLIVNVEKSRISRPKELKFLGFGYYYDANNNNYKVKPHPSSVQKFQRKLRQLTKRNWNVPLAYRILKLNQVIVGWVNYFRVANMKKTTERIDTKLRSRIRVIIWKQWKVAKKQIKSLIRLGIPEEEAKGLTYCRKGYRYIGLSKVVQRAISNKRLKQRGVPSALERYLKVHTVI

SEQ ID NO: 37 - protein, 427 aa, synthetic construct
  REGION 1..427: note = Synthetic construct
MYGETLLDKILDTENLNQAYKKVKRNKGSAGTDGMTVQELGAYIALNKKELISQIRQRKYQPQPVLRVEIPKPDGGIRLLGIPTVKDRLVQQAIAQVLTPMFDKKFSEHSYGFRPNRYAEMAIIQTLEYLNDGHEWIVDIDLERFFDTVNHDRLMNLISRTIQDGDIISLIRKFLVSGVQIDEDYKETVIGTPQGGNLSPLLSNIMLNELDTELESRGLRFVRYADDCIIMVKSEMAARRVMRSVTRFIEEKLGLIVNTTKTKVTRPNDPNMKFLGFGFFKDPQVEVYKAKPHQKSVDNFKFKLKQLTRKNWSVETKFQVERINQVVRGWVNYFKIGFMKKALERIDSHTRFRLRMCIWKKWKTSKNRRKNLIKLGMDRHTAYKYSYSSKGAVRIAYSWVLTKTITNKRLTQFGLLSGVQHYRKVHA

SEQ ID NO: 38 - protein, 427 aa, synthetic construct
  REGION 1..427: note = Synthetic construct
MDTSSLMEQILSKDNLNTAYLQVVRNKGAEGVDGMKYTELKEHLAKNVEIIKEQLRTRKYKPQPVHRVEISKPDGGVRNLGVPTVTDRFVQQAIAQVLTPIYEKQFHDHSYGFRPNRCAQQAIITALDMMNDGYDWIVDIDLEKFFDTVNHDKLMTLIGKTIKDGDVISIIRKFLVSGIMVDDEYRESVIGTPQGGNLSPLLANIILNELDKEMEQRGLNFVRYADDCIIMVGSEMSARRVMRNLTKFIEEKLGLKVNMTKSKVDRPRGLKYLGFGFYFDSRTHQYKAKPHAKSVARFKARMKQLTCRSWGVSNSYKVQKLNELIRGWINYFKIGSMKTLCAKLDSNIRYRLRMCIWKHWKTPQNRAKNLMKLGIEKNRAFHVAYAGYRIAYVCNKGAVNVAISNKRLTQFGLVSMLDYYTKRCVTC

SEQ ID NO: 39 - protein, 427 aa, synthetic construct
  REGION 1..427: note = Synthetic construct
MDTSSLMEQILSKENLNTAYLQVARNKGAEGVDDMKYTELKEHLEKHGETIKEQLRARKYKPQPVRRVEIPKPDGGVRNLGVATVTDRFVQQAIAQVLTPIYEEQFHDHSYGFRPNRCAQQAIITALDMMNDGSAWIVDIDLEKFFDTVNHDKLMTLIGRTIKDGDVISIIRKFLVSGIMDDDEYKESVIGTPQGGNLSPLLANIMLNELDKEMEQRGLNFVRYADDCIIMVGSEMSAKRVMRNLTKFIEEKLGLKVNMSKSKVDRPSGLKYLGFGFYFDSRAHQYKAKPHAKSVAKFKARMKQITCRSWGVGNDYKVKKLNELIRGWINYFKIGSMKTLCAKMDNNIRYRLRMCIWKHWKTPQNRAKNLIKLGVPGWSAWKMAYLHGYAKPARCRDVHQAINNKRLASFGLISMLDYYTERCYLLS

SEQ ID NO: 40 - protein, 425 aa, synthetic construct
  REGION 1..425: note = Synthetic construct
MNTENLLKQILHPNNLNQAYLQVKRNKGAAGVDGMTINELGHYLKENGEEIKDQIRTRSYQPKPVKRIEIPKADGGVRNLGVPTVVDRFIQQAMAQVLTPIYEEKFHENSYGFRPGRCAEMAIIKSLEFMNDGYTWIVDIDLEKFFDKVNHDKLMRLISNTIKDGDVISLIRKFLVSGVMMDDEYKESVIGTPQGGNLSPLLSNIMLNELDQELEARGLNFVRYADDCLILVKSEKAANRVMKSMTKYLEETLGLKVNVTKSKVERPSGIKFLGFGFFWDKNAYQFKAKPHQISIMRVKEKLKRLTRRSWSVSFDYRLKKLKQLIIGWVNYFKIAKMRTVCGNLDKNIRFRLRMCIWKQWKKVQTKYRSLMRLGIDKDKAWEWANTRKGYARVARSFILCRTITNERLKRRGLVSLLDHYQTVHI

SEQ ID NO: 41 - protein, 427 aa, synthetic construct
  REGION 1..427: note = Synthetic construct
MYEGKLLDKILDIDNLNQAFKQVKRNKGAAGVDGMTVQELGAYMALNKDEIISQIRQRTFNPQPVLRVEIPKPNGGVRLLGIPTVKDRVIQQAIAQILTPMFDKTFSEYSYGFRPNRYAEMAIIQTLDYLNDGHDWIVDIDLERFFDTVNHDRLMNLVSRTVDDGDVISLIRKFLVSGVQIDEEYKETIIGTPQGGNLSPLLSNIMLNELDIELEGRGLRFVRYADDCIIMVKSEMAAKRVMRSVTKFIEEKLGLIVNSTKTKVTRPNDPNMKFLGFGFFKDYQSDLYKAKPHQKSVENFQYKLKQLTRKNWSVETKFQVQRINQVIRGWVNYFKVGYMKTVLGKIDAHIRVRLRTCIWKKWKTAKNRRKNLIKLGMERYNAYKYSHTSKGAVRIAYSWVLSTTITNKRLARFGLISCVQHYNKVHA

SEQ ID NO: 42 - protein, 426 aa, synthetic construct
  REGION 1..426: note = Synthetic construct
MDTSSLIEQILSSKNLNEAYLQVFRNKGAEGVDGMKFTELKEHLVKNGEEIKEQLRSRKYKPQPVRRVEIPKPDGGVRNLGVPTVTDRFIQQAIAQVLTPIYEEQFHDHSYGFRPNRCAQQAIMTALDMMNDGNTWIVDIDLEKFFDTVNHDKLMTIIGRTIKDGDIISIVRKFLVIGIMVDNEYEESVIGTPQGGNLSPLLANIMLNELDKEMEKRGLNFVRYADDCIVMVGSEMSANRVMRNLTRFIEEKLGLKVNMTKSKVGRPQGLKYLGFGFYFDSHAHGYKVKPHAKSVEKFKVRMKQLTRRNWGVSNSYKVEKLNQLIKGWINYFRIGEMKWICKDMDAKIRRRLRMCIWVHWKTPENRAKNLMKLGMYRQKAYAIAYSGSRVARLSEGALNYVITNQRLTTFGLVSMLDYYTDRCVTC

SEQ ID NO: 43 - protein, 427 aa, synthetic construct
  REGION 1..427: note = Synthetic construct
MDTSNLMEQILSSDNLNRAYLQVVRNKGAEGVDGMKYTELKEHLAKNGETIKGQLRTRKYKPQPARRVEIPKPDGGVRNLGVPTVTDRFIQQAIAQVLTPIYEEQFHDHSYGFRPNRCAQQAILTALNIMNDGNDWIVDIDLEKFFDTVNHDKLMTLIGRTIKDGDVISIVRKYLVSGIMIDDEYEDSIVGTPQGGNLSPLLANIMLNELDKEMEKRGLNFVRYADDCIIMVGSEMSANRVMRNISRFIEEKLGLKVNMTKSKVDRPSGLKYLGFGFYFDPRAHQFKAKPHAKSVAKFKKRMKELTCRSWGVSNSYKVEKLNQLIRGWINYFKIGSMKTLCKELDSRIRYRLRMCIWKQWKTPQNQEKNLVKLGIDRNTARRVAYTGKRIAYVCNKGAVNVAISNKRLASFGLISMLDYYIEKCVTC

SEQ ID NO: 44 - protein, 564 aa, synthetic construct
  REGION 1..564: note = Synthetic construct
MPPCYPTMTVDQTTGAVTNQTETSWHSINWTKANREVKRLQVRIAKAVKEGRWGKVKALQWLLTHSFYGKALAVKRVTDNSGSRTPGVDGITWSTQEQKTQAIKSLRRRGYKPQPLRRVYIPKANGKQRPLGIPTMKDRAMQALYALALEPVAETTADRNSYGFRRGRCTADAAGQCFLALAKAKSAEHVLDADISGCFDNISHEWLLANTPLDKGILRKWLKSGFVWKQQLFPTHAGTPQGGVISPVLANITLDGMEELLAKHLRGQKVNLIRYADDFVVTGKDEETLEKARNLIQEFLKERGLTLSPEKTKIVHIEEGFDFLGWNIRKYNGVLLIKPAKKNVKAFLKKIRDTLRELRTATQEIVIDTLNPIIRGWANYHKGQVSKETFNRVDFATWHKLWRWARRRHPNKPAQWVKDKYFIKNGSRDWVFGMVMKDKNGELRTKRLIKTSDTRIQRHVKIKADANPFLPEWAEYFEKRKKLKKAPAQYRRIRRELWKKQGGICPVCGGEIEQDMLTDIHHILPKHKGGSDDLDNLVLIHANCHKQVHSRDGQHSRSLLKEGL

SEQ ID NO: 45 - protein, 420 aa, synthetic construct
  REGION 1..420: note = Synthetic construct
MALLERILARDNLITALKRVEANQGAPGIDGVSTDQLRDYIRAHWSTIRAQLLAGTYRPAPVRRVGIPKPGGGTRQLGIPTVVDRLIQQAILQELTPIFDPDFSPSSFGFRPGRNAHDAVRQAQGYIQEGYRYVVDMDLEKFFDRVNHDILMSRVARKVKDKRVLKLIRAYLQAGVMIEGVKVQTEEGTPQGGPLSPLLANILLDDLDKELEKRGLKFCRYADDCNIYVKSLRAGQRVKQSIQRFLEKTLKLKVNEEKSAVDRPWKRAFLGFSFTPERKARIRLAPRSIQRLKQRIRQLTNPNWSISMPERIHRVNQYVMGWIGYFRLVETPSVLQTIEGWIRRRLRLCQWLQWKRVRTRIRELRALGLKETAVMEIANTRKGAWRTTKTPQLHQALGKTYWTAQGLKSLTQRYFELRQG

SEQ ID NO: 46 - protein, 604 aa, synthetic construct
  REGION 1..604: note = Synthetic construct
MYAITKECLEKGDVPRFKGLVEIASSDVVIVSAIHKIKSNQGNSTAGTDGKTISDILTLNYDEAINFVKRCFKKYTPNPIRRVHIPKPGKKEKRPLGILTIADRIIQECVRMVIEPILEAQFFQHSYGFRPYRDAKQAIERCVFICNRIGYNWVIEGDIKGFFDNVNHTILIKQLWHMGIRDRRMLMIIKAMLKAGVIKETKINEMGTPQGGIISPLLANVYLHKLDQWITREWEEKKMRNGTTIRTAKYKSLRDHSTITKPEFYVRYADDWILFTNSRGNAEKWKYRIKKYLKENLKLELSDDKTLITNIKKKPMKFLGFKIKMIPHGKGGKYIGYASADTEKIKGKVEQIRKDLRKLKFATNQEWLITDINRINSKIRGIINYYSSAPSVNRDVRPFKEKLKYASYKALKRYGAKWIPANQCYNLAPLYPDRTEQVPAIKINGRWLGIMSIGFATWIKTNQKNQKETPYTAEGRRIRLQNTGKKPLTVRAQWLLDSGYLNLIQGVKSSKIYNFEFFMNRCYAFNRDKGKCKICGDILQPFNTRTHHINTKLPLNEINKVSNLVTVCDKCHTLIHLKDLSDVNLSRLKTNAIRKLEEYRKCVH

SEQ ID NO: 47 - protein, 635 aa, synthetic construct
  REGION 1..635: note = Synthetic construct
MPKKSKTLCVDDLRHAEYYGMQGTFDELYQKSQSGEVFENLMDLILSRDNILLAYRNIKANKGSYTAGTDKKNITDIGSQTPDDVVKRVRFIVTGSEHGYRPKPVRRKDIPKPNGKTRPLGIPCIWDRLIQQCIKQIMEPICEAKFCNNSYGFRPNRSVEHAINRTYTMLQMMNLHYVIEFDIKGFFDNVNHSKLIRQIWSLGIHDKTLIFIIKRILTAPIKMPDNTTVLPNKGTPQGGIISPLLANIVLNELDWWIASQWEENPIAISRGRERIIGKTKVFDKSHGYRIMKNTEMKEMHIIRYADDFRIFCRTKEDAVRTKEAVTAWIEERLKLEVSPEKTRIVNTRKRWSEFLGFKIRVRLKHHKYVVQSAICDKKVEIERAKLVEQAKNIAKPREKKSCLSEIQLYNSMVLGIQNYYQLATCISIDCRELHRRVMTVLTNRLNTETGSMLKHEGGTITQAEKERFGQSKMIRYVSGIDQMIYPIAFIKNKIPMAKRSIVCSYTKEGRAPIHTELNLNQYVLKGLREKISVGHSTEYHDSKISLFSAQKGKCAISGEEFADAEHVAVWLKVPRALGGFERYKNMVLIHKKYLILLQELPQAVIKDLIKTLNITKKMLVKINSLREQANLSAII

SEQ ID NO: 48 - protein, 470 aa, synthetic construct
  REGION 1..470: note = Synthetic construct
MDSKDMQRLQTTQQRGYPLNREMEFQKTTEVHSISSASEDGRNEVQRYTGKMLEMIVERGNMEAAYKRVVANKGSHGVDGMGVDELLPYLKENWATIKQQLLEGKYKPQPVRRVEIPKPDGGKRLLGIPTVLDRLIQQAIAQILNKVYNHTFSDSSYGFRPGRSAKDAIKAAEAYINEGYTWVVDMDLEKFFDRVNHDIIMSKLEKRIGDKRVLKLIRRYLESGVMINGIKVSTEEGTPQGGPLSPLLANIMLDELDKELEKRGHKFCRYADDCNIYVRSRSAGNRVMKSIKKFIESKLKLKVNEAKSAVDRPWRRKFLGFSFYTKENEVRIRIHEKSIKRFKEKVREITNRNKGISMENRIKRLNQITTGWVNYFGLADAKSIMKTLDEWIRRRLRACIWKQWKKIKTKHDNLVKLGVEEQKAWEYANTRKGYWRISNSPILNKTLTNKYFESIGYKSLSQRYLIVHNS

SEQ ID NO: 49 - protein, 637 aa, synthetic construct
  REGION 1..637: note = Synthetic construct
MAVPKKVLKRQILRNIEYYGLQEVFDELYQKSLENRKFKNLMELILMEENIKLAYRNMKKNDGSTTPGIDGKTIEHLAKMTEKEVIELVRNKLEWYTPKAIRRVEIDKGNGKKRPLGIASIEDRLIQQCILQVLEPICEAKFHDRSNGFRPNRGVENALAQAEKLIQSNKLYIVVDIDIKGFFDNVSHGKLLKQLWTIGIQDKKLISIISAMLKGEIAGIGFPEKGTAQGSIISPLLSNVVLNELDWWIASQWEFMPTRHVYKEAIKANGTQSKSKKYRALRSSTLKECFIVRYADDFKIFCRKHKDAVVMFEATKQWLKTRLGLDISPEKSKIVNLKHSYSEFLGFRIKVHKKGKDTKCKPPVDKYVVKSHISEKALKKIKTNAKERIIAIQKTNGSRAGEFAIRDYNSFVMGVQNYYSMATCVNPDMQTLAYEIKTSIKIRLNTRVKRRTNEVLTPYLSERYGKSKELRFINGVPLVPIGYVQHRVPLHKKAVVNKYTAEGRKEIHKQLETVDIERVHELMKNPVSDETVEFNDNCVSLFVAQRGKCAICKLPLTLENMRCIRKIPKSCGGDDKYNNLIIVHKEMERLIKSQDKKEIKRILNKYKLESNQRRKVNTIRKNAGLEEIDVKALDKEL

SEQ ID NO: 50 - RNA, 350 nt, synthetic construct
  misc_feature 1..350: note = Synthetic construct
  source 1..350: mol_type = other RNA
aaaatccgttgaccttaaacggtcgtgtgggttcaagtccctccacccccacgccggaaacgcaatagccgaaaaacaaaaaacaaaaaaacccccctctccctccccccctaacgttactggccgaagccgcttggaataaggccggtgtgcgtttgtctatatgttattttccaccatattgccgtcttttggcaatgtgagggcccggaaacctggccctgtcttcttgacgagcattcctaggggtctttcccctctcgccaaaggaatgcaaggtctgttgaatgtcgtaaaaaaacaaaaaacaaaacggctattatgcgttaccggcgagacgctacggactt

SEQ ID NO: 51 - DNA, 21 bp, synthetic construct
  misc_feature 1..21: note = Synthetic construct
  source 1..21: mol_type = other DNA
tccagaggaactgcttccttc

SEQ ID NO: 52 - RNA, 1289 nt, synthetic construct
  misc_feature 1..1289: note = Synthetic construct
  source 1..1289: mol_type = other RNA
aaaatccgttgaccttaaacggtcgtgtgggttcaagtccctccacccccacgccggaaacgcaatagccgaaaaacaaaaaacaaaaaaacccccctctccctccccccctaacgttactggccgaagccgcttggaataaggccggtgtgcgtttgtctatatgttattttccaccatattgccgtcttttggcaatgtgagggcccggaaacctggccctgtcttcttgacgagcattcctaggggtctttcccctctcgccaaaggaatgcaaggtctgttgaatgtcgtgaaggaagcagttcctctggaagcttcttgaagacaaacaacgtctgtagcgaccctttgcaggcagcggaaccccccacctggcgacaggtgcctctgcggccaaaagccacgtgtataagatacacctgcaaaggcggcacaaccccagtgccacgttgtgagttggatagttgtggaaagagtcaaatggctctcctcaagcgtattcaacaaggggctgaaggatgcccagaaggtaccccattgtatgggatctgatctggggcctcggtgcacatgctttacatgtgtttagtcgaggttaaaaaacgtctaggccccccgaaccacggggacgtggttttcctttgaaaaacacgatgataatatggccacaaccatgggagtcaaagttctgtttgccctgatctgcatcgctgtggccgaggccaagcccaccgagaacaacgaagacttcaacatcgtggccgtggccagcaacttcgcgaccacggatctcgatgctgaccgcgggaagttgcccggcaagaagctgccgctggaggtgctcaaagagatggaagccaatgcccggaaagctggctgcaccaggggctgtctgatctgcctgtcccacatcaagtgcacgcccaagatgaagaagttcatcccaggacgctgccacacctacgaaggcgacaaagagtccgcacagggcggcataggcgaggcgatcgtcgacattcctgagattcctgggttcaaggacttggagcccatggagcagttcatcgcacaggtcgatctgtgtgtggactgcacaactggctgcctcaaagggcttgccaacgtgcagtgttctgacctgctcaagaagtggctgccgcaacgctgtgcgacctttgccagcaagatccagggccaggtggacaagatcaagggggccggtggtgactaaaaaaaacaaaaaacaaaacggctattatgcgttaccggcgagacgctacggactt

SEQ ID NO: 53 - RNA, 1766 nt, synthetic construct
  misc_feature 1..1766: note = Synthetic construct
  source 1..1766: mol_type = other RNA
gggtctagaaataattttgtttaactttaagaaggagatatacatatgaaaatcgaagaaggtaaaggtcaccatcaccatcaccacggatccatggaagacgccaaaaacataaagaaaggcccggcgccattctatcctctagaggatggaaccgctggagagcaactgcataaggctatgaagagatacgccctggttcctggaacaattgcttttacagatgcacatatcgaggtgaacatcacgtacgcggaatacttcgaaatgtccgttcggttggcagaagctatgaaacgatatgggctgaatacaaatcacagaatcgtcgtatgcagtgaaaactctcttcaattctttatgccggtgttgggcgcgttatttatcggagttgcagttgcgcccgcgaacgacatttataatgaacgtgaattgctcaacagtatgaacatttcgcagcctaccgtagtgtttgtttccaaaaaggggttgcaaaaaattttgaacgtgcaaaaaaaattaccaataatccagaaaattattatcatggattctaaaacggattaccagggatttcagtcgatgtacacgttcgtcacatctcatctacctcccggttttaatgaatacgattttgtaccagagtcctttgatcgtgacaaaacaattgcactgataatgaattcctctggatctactgggttacctaagggtgtggcccttccgcatagaactgcctgcgtcagattctcgcatgccagagatcctatttttggcaatcaaatcattccggatactgcgattttaagtgttgttccattccatcacggttttggaatgtttactacactcggatatttgatatgtggatttcgagtcgtcttaatgtatagatttgaagaagagctgtttttacgatcccttcaggattacaaaattcaaagtgcgttgctagtaccaaccctattttcattcttcgccaaaagcactctgattgacaaatacgatttatctaatttacacgaaattgcttctgggggcgcacctctttcgaaagaagtcggggaagcggttgcaaaacgcttccatcttccagggatacgacaaggatatgggctcactgagactacatcagctattctgattacacccgagggggatgataaaccgggcgcggtcggtaaagttgttccattttttgaagcgaaggttgtggatctggataccgggaaaacgctgggcgttaatcagagaggcgaattatgtgtcagaggacctatgattatgtccggttatgtaaacaatccggaagcgaccaacgccttgattgacaaggatggatggctacattctggagacatagcttactgggacgaagacgaacacttcttcatagttgaccgcttgaagtctttaattaaatacaaaggatatcaggtggcccccgctgaattggaatcgatattgttacaacaccccaacatcttcgacgcgggcgtggcaggtcttcccgacgatgacgccggtgaacttcccgccgccgttgttgttttggagcacggaaagacgatgacggaaaaagagatcgtggattacgtcgccagtcaagtaacaaccgcgaaaaagttgcgcggaggagttgtgtttgtggacgaagtaccgaaaggtcttaccggaaaactcgacgcaagaaaaatcagagagatcctcataaaggccaagaagggcggaaagtccaaactcgagtaaggttaacctgcaggagg

SEQ ID NO: 54 - DNA, 22 bp, synthetic construct
  misc_feature 1..22: note = Synthetic construct
  source 1..22: mol_type = other DNA
ttccaattcagcgggggccacc

SEQ ID NO: 55 - RNA, 747 nt, synthetic construct
  misc_feature 1..747: note = Synthetic construct
  source 1..747: mol_type = other RNA
aaaatccgttgaccttaaacggtcgtgtgggttcaagtccctccacccccacgccggaaacgcaatagccgaaaaacaaaaaacaaaaaaacccccctctccctccccccctaacgttactggccgaagccgcttggaataaggccggtgtgcgtttgtctatatgttattttccaccatattgccgtcttttggcaatgtgagggcccggaaacctggccctgtcttcttgacgagcattcctaggggtctttcccctctcgccaaaggaatgcaaggtctgttgaatgtcgttggaggtgctcaaagagatggaagccaatgcccggaaagctggctgcaccaggggctgtctgatctgcctgtcccacatcaagtgcacgcccaagatgaagaagttcatcccaggacgctgccacacctacgaaggcgacaaagagtccgcacagggcggcataggcgaggcgatcgtcgacattcctgagattcctgggttcaaggacttggagcccatggagcagttcatcgcacaggtcgatctgtgtgtggactgcacaactggctgcctcaaagggcttgccaacgtgcagtgttctgacctgctcaagaagtggctgccgcaacgctgtgcgacctttgccagcaagatccagggccaggtggacaagatcaagggggccggtggtgactaaaaaaaacaaaaaacaaaacggctattatgcgttaccggcgagacgctacggactt

SEQ ID NO: 56 - RNA, 350 nt, synthetic construct; identical to SEQ ID NO: 50
  misc_feature 1..350: note = Synthetic construct
  source 1..350: mol_type = other RNA

SEQ ID NO: 57 - DNA, 20 bp, synthetic construct
  misc_feature 1..20: note = Synthetic construct
  source 1..20: mol_type = other DNA
cagcgctcaatcctttggga

SEQ ID NO: 58 - DNA, 22 bp, synthetic construct
  misc_feature 1..22: note = Synthetic construct
  source 1..22: mol_type = other DNA
gacctgccacattgggtcagta

SEQ ID NO: 59 - DNA, 20 bp, synthetic construct
  misc_feature 1..20: note = Synthetic construct
  source 1..20: mol_type = other DNA
tctgtcacggaaaagtcgca

SEQ ID NO: 60 - DNA, 20 bp, synthetic construct
  misc_feature 1..20: note = Synthetic construct
  source 1..20: mol_type = other DNA
tgatccggctacctgtttgt

SEQ ID NO: 61 - DNA, 20 bp, synthetic construct
  misc_feature 1..20: note = Synthetic construct
  source 1..20: mol_type = other DNA
ggagtggttggggtgacttt

SEQ ID NO: 62 - DNA, 20 bp, synthetic construct
  misc_feature 1..20: note = Synthetic construct
  source 1..20: mol_type = other DNA
tcaactgccatacgaagcgt

SEQ ID NO: 63 - DNA, 22 bp, synthetic construct
  misc_feature 1..22: note = Synthetic construct
  source 1..22: mol_type = other DNA
tatgttggtggatcctgttcgg

SEQ ID NO: 64 - DNA, 22 bp, synthetic construct
  misc_feature 1..22: note = Synthetic construct
  source 1..22: mol_type = other DNA
gaccaagacttgtgaggccata

SEQ ID NO: 65 - DNA, 25 bp, synthetic construct
  misc_feature 1..25: note = Synthetic construct
  source 1..25: mol_type = other DNA
ggaaaatgtgataaaaacaaggtgg

SEQ ID NO: 66 - DNA, 22 bp, synthetic construct
  misc_feature 1..22: note = Synthetic construct
  source 1..22: mol_type = other DNA
gactcttgtccaagcatcagga

SEQ ID NO: 67 - DNA, 19 bp, synthetic construct
  misc_feature 1..19: note = Synthetic construct
  source 1..19: mol_type = other DNA
tccctggagaagagctacg

SEQ ID NO: 68 - DNA, 20 bp, synthetic construct
  misc_feature 1..20: note = Synthetic construct
  source 1..20: mol_type = other DNA
gtagtttcgtggatgccaca

SEQ ID NO: 69 - DNA, 21 bp, synthetic construct
  misc_feature 1..21: note = Synthetic construct
  source 1..21: mol_type = other DNA
aaggtgaaggtcggagtcaac

SEQ ID NO: 70 - DNA, 23 bp, synthetic construct
  misc_feature 1..23: note = Synthetic construct
  source 1..23: mol_type = other DNA
ggggtcatttgatggcaacaata

SEQ ID NO: 71 - DNA, 23 bp, synthetic construct
  misc_feature 1..23: note = Synthetic construct
  source 1..23: mol_type = other DNA
ggtggtctcctctgacttcaaca

SEQ ID NO: 72 - DNA, 23 bp, synthetic construct
  misc_feature 1..23: note = Synthetic construct
  source 1..23: mol_type = other DNA
gttgctgtagccaaattcgttgt

SEQ ID NO: 73 - DNA, 27 bp, synthetic construct
  misc_feature 1..27: note = Synthetic construct
  source 1..27: mol_type = other DNA
ccacaaattatgcagtcaagtttccca

SEQ ID NO: 74 - DNA, 24 bp, synthetic construct
  misc_feature 1..24: note = Synthetic construct
  source 1..24: mol_type = other DNA
ccatgatcacgaaggtggttttcc

SEQ ID NO: 75 - DNA, 21 bp, synthetic construct
  misc_feature 1..21: note = Synthetic construct
  source 1..21: mol_type = other DNA
ctaacagggctctccctgagc

SEQ ID NO: 76 - DNA, 20 bp, synthetic construct
  misc_feature 1..20: note = Synthetic construct
  source 1..20: mol_type = other DNA
gttccaagctccggcaaagg

SEQ ID NO: 77 - DNA, 22 bp, synthetic construct
  misc_feature 1..22: note = Synthetic construct
  source 1..22: mol_type = other DNA
tgaagcagctctccctacagtg

SEQ ID NO: 78 - DNA, 22 bp, synthetic construct
  misc_feature 1..22: note = Synthetic construct
  source 1..22: mol_type = other DNA
tggcacaatgttctccagttcc

SEQ ID NO: 79 - DNA, 53 bp, synthetic construct
  misc_feature 1..53: note = Synthetic construct
  source 1..53: mol_type = other DNA
acttgcctgtcgctctatcttctttgttttttccctgcaggttaaccttactc

SEQ ID NO: 80 - DNA, 42 bp, synthetic construct
  misc_feature 1..42: note = Synthetic construct
  source 1..42: mol_type = other DNA
cctgcagggaaaaaacaaagaagatagagcgacaggcaagta

SEQ ID NO: 81 - RNA, 1271 nt, synthetic construct
  misc_feature 1..1271: note = Synthetic construct
  source 1..1271: mol_type = other RNA
ggattctaaaacggattaccagggatttcagtcgatgtacacgttcgtcacatctcatctacctcccggttttaatgaatacgattttgtaccagagtcctttgatcgtgacaaaacaattgcactgataatgaattcctctggatctactgggttacctaagggtgtggcccttccgcatagaactgcctgcgtcagattctcgcatgccagagatcctatttttggcaatcaaatcattccggatactgcgattttaagtgttgttccattccatcacggttttggaatgtttactacactcggatatttgatatgtggatttcgagtcgtcttaatgtatagatttgaagaagagctgtttttacgatcccttcaggattacaaaattcaaagtgcgttgctagtaccaaccctattttcattcttcgccaaaagcactctgattgacaaatacgatttatctaatttacacgaaattgcttctgggggcgcacctctttcgaaagaagtcggggaagcggttgcaaaacgcttccatcttccagggatacgacaaggatatgggctcactgagactacatcagctattctgattacacccgagggggatgataaaccgggcgcggtcggtaaagttgttccattttttgaagcgaaggttgtggatctggataccgggaaaacgctgggcgttaatcagagaggcgaattatgtgtcagaggacctatgattatgtccggttatgtaaacaatccggaagcgaccaacgccttgattgacaaggatggatggctacattctggagacatagcttactgggacgaagacgaacacttcttcatagttgaccgcttgaagtctttaattaaatacaaaggatatcaggtggcccccgctgaattggaatcgatattgttacaacaccccaacatcttcgacgcgggcgtggcaggtcttcccgacgatgacgccggtgaacttcccgccgccgttgttgttttggagcacggaaagacgatgacggaaaaagagatcgtggattacgtcgccagtcaagtaacaaccgcgaaaaagttgcgcggaggagttgtgtttgtggacgaagtaccgaaaggtcttaccggaaaactcgacgcaagaaaaatcagagagatcctcataaaggccaagaagggcggaaagtccaaactcgagtaaggttaacctgcagggaaaaaacaaaaaacaaaacggctattatgcgttaccggcgagacgctacggactt

SEQ ID NO: 82 - DNA, 50 bp, synthetic construct
  misc_feature 1..50: note = Synthetic construct
  source 1..50: mol_type = other DNA
acttgcctgtcgctctatctttgttttttccctgcaggttaaccttactc

SEQ ID NO: 83 - RNA, 84 nt, synthetic construct
  misc_feature 1..84: note = Synthetic construct
  source 1..84: mol_type = other RNA
rtrgrargrgrtrargrtrargrgrtrtrgrtrartrargrtrtrtrarcrtrgrarcrcrargrgrarcrgrarcrgrarcra

SEQ ID NO: 84 - RNA, 40 nt, synthetic construct
  misc_feature 1..40: note = Synthetic construct
  source 1..40: mol_type = other RNA
rtrarcrtrgrarcrcrargrgrarcrgrarcrgrarcra

SEQ ID NO: 85 - RNA, 26 nt, synthetic construct
  misc_feature 1..26: note = Synthetic construct
  misc_feature 21..26: note = n is a, c, g, or u
  source 1..26: mol_type = other RNA
tgtcgtcgtcctggtcagtannnnnn

SEQ ID NO: 86 - DNA, 20 bp, synthetic construct
  misc_feature 1..20: note = Synthetic construct
  source 1..20: mol_type = other DNA
tgtcgtcgtcctggtcagta

SEQ ID NO: 87 - DNA, 20 bp, synthetic construct
  misc_feature 1..20: note = Synthetic construct
  source 1..20: mol_type = other DNA
tactgaccaggacgacgaca